European Patent Application EP 4 785 779 A1, published August 5, 2026. Title: A plant with altered flower color and a method for creating the same. Applicant: サントリーフラワーズ株式会社. The sequence listing filed with the application follows.

SEQUENCE LISTING (15 sequences)

SEQ ID NO: 1 - DNA, 16 bp, Mandevilla
  source 1..16: mol_type = genomic DNA
gtatcttgaacaatta

SEQ ID NO: 2 - DNA, 30 bp, Mandevilla
  source 1..30: mol_type = genomic DNA
atatataattattagttagggattaaagag

SEQ ID NO: 3 - DNA, 173 bp, Mandevilla
  source 1..173: mol_type = genomic DNA
ttagtgtctcttccttagttcctgattagtttgtgtatatttttcaatttagttcctgattagtttgtgcatatttttcaatttacatacttaacgtattatgaacgatctcttaaaattcagaattaattgaatgaaacttaaatggctgaattataaaaataaaaaaaaaa

SEQ ID NO: 4 - DNA, 1374 bp, Mandevilla
  source 1..1374: mol_type = genomic DNA
atggccaccaaaaacttatgtgaaaagcatgttgctgttcttacatttccatttgcatcccatcctggccttctgttaggccttctacatagattagttaaggctgcaccacatgtgactttctcttttctcagcactgccaagtccaatgctttattgttttctaccaaaacacgggcagatcaaaatatcaaggcctttgatgtgccggatggggtgcccgaaggacatgtttttctgggcaagccagctgaggatattgacctgttcttgaaggtggcagaggaagttttcaagaaaggtgtcgaagaggctgagaaggtaatagggatgaaggttagctgcgtgatggcagatgcgtttctatggttttctgctgggatggctgaggaattaagtgttccttggattcctgtttggacatctggagctagctccctctctgttcatgtgtacacagaattgatcaggcaaactgttggaattgacggtatagctggccgtgaagatgaaattcttacattcgttcctggtttttctgaacttcggcttggtgatttgcctagcggagttgtgtatggaaggctggattcacctttctcagtcatgctatataaaatgggaaataatttacatcgagcagatgctttgcctatgaattcctttgaagaattggaccctcccatcacgaaagatctgaagtccaagtttgaaaatgctctttacattggcccctttaatttgacatctccaccaccaatagcaaacttcccagatacacatggttgcattccatggttagaccgacatgaaaaacggaccgttgcatacattgcctttggaaccgtggcaacactaccgccccaggagttgaaggcactggctgaagctcttgaagcaactaatactccatttatttggtcacttaaagacaacatgaaaactcatctacctgaaggattcttggaaagaacaagtgagacaggcaaaatagttccatgggcagctcaagagaaaatattagcacatgagtctgtgggagttttcttgaaccattgtggttggaattcagtgatggaaagcgttgctgctggtgtgcctataattggcaggccatttttcggggatcatcaactcaacacttggatggtcgagaaagtctggaaaattggggtgagaattgagggtggtttgtttacaaaagatgctacaattagagctcttgaattggttttgaagcaggaagaagggcagaggttaaaggatcagattgttacttatgaaaagcttgctctagaggctgtgcaaccaaatggatcctcaactagaaacttagaatctttgatacggattattgctgatggtaaggcttga

SEQ ID NO: 5 - protein, 457 aa, Mandevilla
MATKNLCEKHVAVLTFPFASHPGLLLGLLHRLVKAAPHVTFSFLSTAKSNALLFSTKTRADQNIKAFDVPDGVPEGHVFLGKPAEDIDLFLKVAEEVFKKGVEEAEKVIGMKVSCVMADAFLWFSAGMAEELSVPWIPVWTSGASSLSVHVYTELIRQTVGIDGIAGREDEILTFVPGFSELRLGDLPSGVVYGRLDSPFSVMLYKMGNNLHRADALPMNSFEELDPPITKDLKSKFENALYIGPFNLTSPPPIANFPDTHGCIPWLDRHEKRTVAYIAFGTVATLPPQELKALAEALEATNTPFIWSLKDNMKTHLPEGFLERTSETGKIVPWAAQEKILAHESVGVFLNHCGWNSVMESVAAGVPIIGRPFFGDHQLNTWMVEKVWKIGVRIEGGLFTKDATIRALELVLKQEEGQRLKDQIVTYEKLALEAVQPNGSSTRNLESLIRIIADGKA

SEQ ID NO: 6 - DNA, 1425 bp, Mandevilla
  source 1..1425: mol_type = genomic DNA
atggagtacgagtacgcgtacgactgcgaaaattgcttgagcattgtgatgtacccatggtttggaatgggacatctcacggcatttcttcatctgtccaataagcttgctcagataggccataaaattttcttcattttgccaacaaaatcgcaatccaagttggaaaacttcaatcttcatccacaccgcatcaagttcatacctctgactgttccaaaagttgaaggccttccgtctgatgctgaaacaacttcagatatgccttcttcaatgcaacctcttcttcgacttgccatggatcaaacacagctaactattgaatctttactccaagacattcgaccgcattttgtcttctatgattttcagtattggttgccgtcggtagcacgccctttaggcataaaggcggttcatttttgcattataagccctgcaacaataggttattcctgcatccgcgaggaccagatgaaagatgctcatgaactgatgaaacctccctctagttatccttcatccagcgtcaagcttcatgcccatgaagctcgaggactatttttcactagaaacacgaaagagattgcgagcggcatgtcactcttgaagcgggttttcatctccatttctgaatctgatgccattggcttcaaaacatgtagagaaatggaagggccttactgtgaatttctagaaaaaaagctcaagaaaccagtcattctggctggaccggtggttcctgtaccgccatcttctgctctagaagaaacatggcaaaagtggctgaacgggttcagagccaaaacagttattttctgtgcatttggaagtgaatgcattcttaaaaaggatcaatttcaagaactgttgttgggttttgagcttacaggtctaccatttctagtcgctcttaaaccacctgtcggtgctgagacagctgaagaagctctaccagaaggtttcaaagagagaacaaaagaaagaggtgttgttcatgaaggttgggtgcagcaacagctgattttagctcacccttctgtgggatgttttgtctcccactgtggatcagggtcaatatcagaagccttggtgagtgattgccaaatggttctcttgccccatattggtgatcaagttatcaatgcaagagtgatgggtgcagatctcaaagttggagttgaagtggaaaaaggagatgaagatgggctgtttacgaaagaaactgtctgcagagctataagattggtgatggatgaagacagtgagattgggaaggaagtaagagcaaaccataccaaatggagggacttcttgttgcgtgaagggcttgaaactagttatgttgatgaatttgtgcttaacctacgaaaattattgggcgccgatcagaacaatggtagcgcaatgcatcatccatgttaa

SEQ ID NO: 7 - protein, 474 aa, Mandevilla
MEYEYAYDCENCLSIVMYPWFGMGHLTAFLHLSNKLAQIGHKIFFILPTKSQSKLENFNLHPHRIKFIPLTVPKVEGLPSDAETTSDMPSSMQPLLRLAMDQTQLTIESLLQDIRPHFVFYDFQYWLPSVARPLGIKAVHFCIISPATIGYSCIREDQMKDAHELMKPPSSYPSSSVKLHAHEARGLFFTRNTKEIASGMSLLKRVFISISESDAIGFKTCREMEGPYCEFLEKKLKKPVILAGPVVPVPPSSALEETWQKWLNGFRAKTVIFCAFGSECILKKDQFQELLLGFELTGLPFLVALKPPVGAETAEEALPEGFKERTKERGVVHEGWVQQQLILAHPSVGCFVSHCGSGSISEALVSDCQMVLLPHIGDQVINARVMGADLKVGVEVEKGDEDGLFTKETVCRAIRLVMDEDSEIGKEVRANHTKWRDFLLREGLETSYVDEFVLNLRKLLGADQNNGSAMHHPC

SEQ ID NO: 8 - DNA, 1368 bp, Mandevilla
  source 1..1368: mol_type = genomic DNA
atggccaccaaaaacttatgtgaaaagcatgttgctgttcttacatttccatttgcatcccatcctggccttctgttaggccttctacatagattagttaaggctgcaccacatgtgactttctcttttctcagcactgccaagtccaatgctttattgttttctgccaaaacaccggcagatcaaaatatcaaggcctttgatgtgccggatggggtgcccgaaggacatgtttttctgggcaagccagctgaggatattgacctgttcttgaaggtggcagaggatgttttcaagaaaggtgtggaagaggctgagaaggtaatagggatgaaggttagctgcgtgatggcagatgcgtttctatggttttctgctgggatggctgaggaattaagtgttccttggattcctgtttggacatctggagctagctccctctctgttcatgtgtacacggaattgatcaggcaaactgttggaattgacggtatagctggccgtgaagatgaaattcttacattcgttcctggtttttctgaacttcggcttggtgatttgcctagcggtgttgtgtatggaaggctggattcgcctttctcagtcatgctatataaaatgggaaaaaatttacatcgagcagatgctttgcctttgaattcctttgaagaattggaccctcccatcacgaaagatctgaagtccaagtttaaaaatgctctttacattggcccctttaacttgacatctcccccaccaatagcaaatttcccagatacacatggttgcattccatggttagaccgacatgaaaaacgaaccgttgcatacattgcctttggaaccgtggcaacaccaccgccccacgagttgaaggcactggctgaagctcttgaagcaactaatactccatttatttggtcacttaaagacaacatgaaaactcatctacctgaaggattcttggaaagaacaagtgagacaggcaaaatagttccttgggcagcccaagagcaaatattagcacatgagtctgtgggagttttcttgagccattgtggttggaattcagtgatggaaagcgttgctgcaggtgtgcctataattggcaggccattttttggggatcatcaactcaacacttggatggtcgagaaagtctggaaaattggggtgagaattgagggtggtttgtttacaaaagatgctacaattagagctcttgaattggttttgaagcaggaagaagggcagaggttaaaggatcagattgttacttatgaaaagcttgctctagaggctgtggaaccaaatgaatcctcaactagaaacttagaatctttgatacggattattgctgatggttaa

SEQ ID NO: 9 - DNA, 1368 bp, Mandevilla
  source 1..1368: mol_type = genomic DNA
atggccaccaaaaacttatgtgaaaagcatgttgctgttcttacatttccatttgcatcccatcctggccttctgttaggccttctacatagattagttaaggctgcaccacatgtgactttctcttttctcagcactgccaagtccaatgctttattgttttctgccaaaacaccggcagatcaaaatatcaaggcctttgatgtgccggatggggtgcccgaaggacatgtttttctgggcaagccagctgaggatattgacctgttcttgaaggtggcagaggatgttttcaagaaaggtgtggaagaggctgagaaggtaatagggatgaaggttagctgcgtgatggcagatgcgtttctatggttttctgctgggatggctgaggaattaagtgttccttggattcctgtttggacatctggagctagctccctctctgttcatgtgtacacggaattgatcaggcaaactgttggaattgacggtatagctggccgtgaagatgaaattcttacattcgttcctggtttttctgaacttcggcttgttgatttgcctagcggtgttgtgtatggaaggctggattcgcctttctcagtcatgctatataaaatgggaaaaaatttacatcgagcagatgctttgcctttgaattcctttgaagaattggaccctcccatcacgaaagatctgaagtccaagtttaaaaatgctctttacattggcccctttaacttgacatctcccccaccaatagcaaatttccccgatacacatggttgcattccatggttagaccgacatgaaaaacgaaccgttgcatacattgcctttggaaccgtggcaacaccaccgccccacgagttgaaggcactggctgaagctcttgaagcaactaatactccatttatttggtcacttaaagacaacatgaaaactcatctacctgaaggattcttggaaagaacaagtgagacaggcaaaatagttccttgggcagctcaagagcaaatattagcacatgagtctgtgggagttttcttgagccattgtggttggaattcagtgatggaaagcgttgctgcaggtgtgcctataattggcaggccattttttggggatcatcaactcaacacttggatggtcgagaaagtctggaaaattggggtgagaattgagggtggtttgtttacaaaagatgctacaattagagctcttgaattggttttgaagcaggaagaagggcagaggttaaaggatcagattgttacttatgaaaagcttgctctagaggctgtggaaccaaatggatcctcaactagaaacttagaatctttgatacggattattgctgatggttaa

SEQ ID NO: 10 - DNA, 1419 bp, Mandevilla
  source 1..1419: mol_type = genomic DNA
atggagtacgagtacgactgcgaaaattgcttgagcattgtgatgtacccatggtttggaatgggacatctcacggcatttcttcatctgtccaataagcttgctcagaaaggccatagaattttcttcattttgccaacaaaatcgcaatccaagttggaaaacttcaatcttcatccacaccgcatcaagttcatacctctgactgttccaaaagttgaaggccttccatctgatgctgaaacaacttcagatgtgccttcttcaatgcaatctcttcttcgacttgccatggatcaaacacagccaactattgaatctttactccaagacattcgaccgcatttcgtcttctatgattttcaatattggttgccgtcggtagcacgccctttaggcataaaggcggttcatttttgcattataagccctgcaactataggttattcctgcatccgccaggaccagatgacagatgctcatgaactgatgaaacctccctctagttatccttcatccagcgtcaagcttcatgcccatgaagctcgaggactatttttcactagaaacacgaaagagattgggagcggcatgtcactcttgaagcgggttttcatctccatttctgaatctgatgccattggcttcaaaacatgtggagaaatagaagggccttactgtgaatttctagaaaaaaagctcatgaaaccagtcattctggctggaccggtggttcctgtaccaccatcttctactctagaagaaacatggcaaaagtggctgaacgggttcagagccaaaacagttattttctgtgcatttggaagtgaatgcattcttaaaaaggatcaatttcaagaactgttgttgggttttgagcttacaggtctaccatttctagtcgctctgaaaccacctgtcggtgctgagacagttgaagaagctctaccagaaggtttcaaagagagaacacaagaaagaggtgttgttcatggaggttgggtgcagcaacagctgattttatctcacccttctgtgggatgttttgtctcccactgtggatcagggtcaatatcagaagccttggtgagtgattgccaaatggttctcttgccccatattggtgatcaagttatcaatgcaagaatgatgggtgcagatctcaaagttggagttgaagtggaaaaaggagatgaagatgggctgtttacgaaagaaagtgtctgcagagctataagattggtgatggatgaagacagtgagattgggaaggaagtaagagcaaaccataccaaatggagggacttcttgttgcgtgaggggctcgaaactagttatgttgatgaatttgttcttaacctacgaaaattattgggcaccgatcagaacaatggtagcgcaatgcatcatccatgttaa

SEQ ID NO: 11 - DNA, 1419 bp, Mandevilla
  source 1..1419: mol_type = genomic DNA
atggagtaccagtacgactgcgaaaattgcttgagcattgtgatgtacccatggtttggaatgggacatctcacggcatttcttcatctgtccaataagcttgctcagaaaggccatagaattttcttcattttgccaacaaaatcgcaatccaagttggaaaacttcaatcttcatccacaccgcatcaagttcatacctctgactgttccaaacgttgaaggccttccatctgatgctgaaacaacttcagatgtgccttcttcaatgcaacctcttcttcgacttgccatggatcaaacacagccaactattgaatctttactccaagacattcgaccgcatttcgtcttctatgattttcagtattggttgccgtcggtagcacgccctttaggcataaaggcggttcatttttgcattataagccctgcaactaaaggttattcctgcatccgccaggaccggatgaaagatgctcatgaactgatgaaacctccctctagttatccttcatccagcgtcaagcttcatgcccatgaagcgcgaggactatttttcactagaaacacgaaagagattgggagcggcatgtcactcttgaagcgggttttcatctccatttctgaatctgatgccattggcttcaaaacatgtggagaaatagaagggccttactgtgaatttctagaaaaaaagctcatgaaaccagtcattctggctggaccggtggttcctgtaccaccatcttctactctagaagaaacatggcaaaagtggctgaacgggttcagagccaaaacagttattttctgtgcatttggaagtgaatgcattcttaaaaaggatcaatttcaagaactgttgttgggttttgagcttacaggtctaccatttctagtcgctctgaaaccacctgtcggtgctgagacagttgaagaagctctaccagaaggtttcaaagagagaacacaagaaagaggtgttgttcatggaggttgggtgcagcaacagctgattttatctcacccttctgtgggatgttttgtctcccactgtggatcagggtcaatatcagaagccttggtgagtgattgccaaatggttctcttgccccatattggtgatcaagttatcaatgcaagaatgatgggtgcagatctcaaagttggagttgaagtggaaaaaggagatgaagatgggctgtttacgaaagaaactgtctgcaaagctataagattggtgatggatgaagacagtgagattgggaaggaagtaagagcaaaccataccaaatggagggacttcttgttgcgtgaagggctcgaaactagttatgttgatgaatttgttcttaacctacgaaaattattgggcaccgatcagaacaatggtagcgcaatgcatcatccatgttaa

SEQ ID NO: 12 - DNA, 19 bp, Mandevilla
  source 1..19: mol_type = genomic DNA
actggcctcgccattaacg

SEQ ID NO: 13 - DNA, 29 bp, Mandevilla
  source 1..29: mol_type = genomic DNA
gtaatttaattaagatgcgtaattctctg

SEQ ID NO: 14 - DNA, 22 bp, Mandevilla
  source 1..22: mol_type = genomic DNA
agtgtctcttccttagttcctg

SEQ ID NO: 15 - DNA, 29 bp, Mandevilla
  source 1..29: mol_type = genomic DNA
ctgaattttaagagatcgttcataatacg